European Patent Specification EP 2 995 315 B1, published December 27, 2023. Title: COMPOSITIONS AND METHODS FOR TREATING HEMATOLOGIC CANCERS TARGETING THE SIRP.ALPHA - CD47 INTERACTION. Applicant: University Health Network Hospital for Sick Children Dick, John Jin, Liqing Prasolova, Tatiana Theocharides, Alexandre Danska, Jayne Wang, Jean C. Y. The sequence listing filed with the application follows.

SEQUENCE LISTING (13 sequences)

SEQ ID NO: 1 - protein, 507 aa, mouse
MEPAGPAPGRLGPLLLCLLLSASCFCTGATRTEVKVIQPEKSVSVAAGDSTVLNCTLTSLLPVGPIRWYRGVGQSRQLIYSFTTEHFPRVTNVSDATKRSNLDFSIRISNVTPEDAGTYYCVKFQRGSPDTEIQSGGGTEVYVLAKPSPPEVSGPADRGIPDQKVNFTCKSHGFSPRNITLKWFKDGQELHPLETTVNPSGKNVSYNISSTVRVVLNSMDVHSKVICEVAHITLDRSPLRGIANLSNFIRVSPTVKVTQQSPTSMSQVNLTCRAERFYPEDLQLIWLENGNVSRNDTPKNLTKNTDGTYNYTSLFLVNSSAHREDVVFTCQVKHDQQPAITRNHTVLGLAHSSDQGSMQTFPGNNATHNWNVFIGVGVACALLVVLLMAALYLLRIKQKKAKGSTSSTRLHEPEKNAREITQIQDTNDINDITYADLNLPKEKKPAPRAPEPNNHTEYASIETGKVPRPEDTLTYADLDMVHLSRAQPAPKPEPSFSEYASVQVQRK

SEQ ID NO: 2 - protein, 509 aa, mouse
MEPAGPAPGRLGPLLLCLLLSASCFCTGATGKELKVTQPEKSVSVAAGDSTVLNCTLTSLLPVGPIRWYRGVGPSRLLIYSFAGEYVPRIRNVSDTTKRNNMDFSIRISNVTPADAGIYYCVKFQKGSSEPDTEIQSGGGTEVYVLAKPSPPEVSGPADRGIPDQKVNFTCKSHGFSPRNITLKWFKDGQELHPLETTVNPSGKNVSYNISSTVRVVLNSMDVNSKVICEVAHITLDRSPLRGIANLSNFIRVSPTVKVTQQSPTSMNQVNLTCRAERFYPEDLQLIWLENGNVSRNDTPKNLTKNTDGTYNYTSLFLVNSSAHREDVVFTCQVKHDQQPAITRNHTVLGFAHSSDQGSMQTFPDNNATHNWNVFIGVGVACALLVVLLMAALYLLRIKQKKAKGSTSSTRLHEPEKNAREITQIQDTNDINDITYADLNLPKEKKPAPRAPEPNNHTEYASIETGKVPRPEDTLTYADLDMVHLSRAQPAPKPEPSFSEYASVQVQRK

SEQ ID NO: 3 - protein, 513 aa, mouse
MEPAGPAPGRLGPLLLCLLLSASCFCTGATGKELKVTQPEKSVSVAAGDSTVLNCTLTSLLPVGPIRWYRGVGPSRLLIYSFAGEYVPRIRNVSDTTKRNNMDFSIRISNVTPADAGIYYCVKFQKGSSEPDTEIQSGGGTEVYVLAKPSPPEVSGPADRGIPDQKVNFTCKSHGFSPRNITLKWFKDGQELHPLETTVNPSGKNVSYNISSTVRVVLNSMDVNSKVICEVAHITLDRSPLRGIANLSNFIRVSPTVKVTQQSPTSMNQVNLTCRAERFYPEDLQLIWLENGNVSRNDTPKNLTKNTDGTYNYTSLFLVNSSAHREDVVFTCQVKHDQQPAITRNHTVLGFAHSSDQGSMQTFPDNNATHNWNVFIGVGVACALLVVLLMAALYLLRIKQKKAKGSTSSTRLHEPEKNAREITQVQSLIQDTNDINDITYADLNLPKEKKPAPRAPEPNNHTEYASIETGKVPRPEDTLTYADLDMVHLSRAQPAPKPEPSFSEYASVQVQRK

SEQ ID NO: 4 - protein, 120 aa, human
GVAGEEELQVIQPDKSVLVAAGETATLRCTATSLIPVGPIQWFRGAGPGRELIYNQKEGHFPRVTTVSDLTKRNNMDFSIRIGNITPADAGTYYCVKFRKGSPDDVEFKSGAGTELSVRA

SEQ ID NO: 5 - protein, 119 aa, human
GVAGEEELQVIQPDKSVSVAAGESAILHCTVTSLIPVGPIQWFRGAGPARELIYNQKEGHFPRVTTVSESTKRENMDFSISISNITPADAGTYYCVKFRKGSPDTEFKSGAGTELSVRA

SEQ ID NO: 6 - protein, 120 aa, human
GVAGEEELQVIQPDKSVSVAAGESAILHCTVTSLIPVGPIQWFRGAGPARELIYNQKEGHFPRVTTVSESTKRENMDFSISISNITPADAGTYYCVKFRKGSPDDVEFKSGAGTELSVRA

SEQ ID NO: 7 - protein, 120 aa, human
GVAGEEELQVIQPDKSVLVAAGETATLRCTATSLIPVGPIQWFRGAGPGRELIYNQKEGHFPRVTTVSDLTKRNNMDFSIRISNITPADAGTYYCVKFRKGSPDDVEFKSGAGTELSVRA

SEQ ID NO: 8 - protein, 119 aa, mouse
ATGKELKVTQPEKSVSVAAGDSTVLNCTLTSLLPVGPIRWYRGVGPSRLLIYSFAGEYVPRIRNVSDTTKRNNMDFSIRISNVTPADAGIYYCVKFQKGSSEPDTEIQSGGGTEVYVLA

SEQ ID NO: 9 - protein, 119 aa, mouse; identical to SEQ ID NO: 8

SEQ ID NO: 10 - protein, 117 aa, mouse
ATRTEVKVIQPEKSVSVAAGDSTVLNCTLTSLLPVGPIRWYRGVGQSRQLIYSFTTEHFPRVTNVSDATKRSNLDFSIRISNVTPEDAGTYYCVKFQRGSPDTEIQSGGGTEVYVLA

SEQ ID NO: 11 - protein, 119 aa, mouse
ATGTEVKVTQPEKSVSVAAGDSTILNCTVTSLLPVGPIRWYRGVGQSRLLIYSFTGEHFPRVRNVSDTTKRNNMDFSIRISNVTPEDAGTYYCVKFQRGSSEPDTEIQSGGGTEVYVLA

SEQ ID NO: 12 - protein, 119 aa, mouse
VTGKELKVTQPEKSVSVAAGDSTVLNCTLTSLLPVGPIKWYRGVGQSRLLIYSFTGEHFPRVTNVSDATKRNNMDFSIRISNVTPEDAGTYYCVKFQKGPSEPDTEIQSGGGTEVYVLA

SEQ ID NO: 13 - protein, 368 aa, human
MEPAGPAPGRLGPLLCLLLAASCAWSGVAGEEELQVIQPDKSVSVAAGESAILHCTVTSLIPVGPIQWFRGAGPARELIYNQKEGHFPRVTTVSESTKRENMDFSISISNITPADAGTYYCVKFRKGSPDTEFKSGAGTELSVRPPCPSCPAPEFLGGPSVFLFPPKPKDTLMISRTPEVTCVVVDVSQEDPEVQFNWYVDGVEVHNAKTKPREEQFNSTYRVVSVLTVLHQDWLNGKEYKCKVSNKGLPSSIEKTISKAKGQPREPQVYTLPPSQEEMTKNQVSLTCLVKGFYPSDIAVEWESNGQPENNYKTTPPVLDSDGSFFLYSRLTVDKSRWQEGNVFSCSVMHEALHNHYTQKSLSLSPGK